European Patent Specification EP 3 426 805 B1, published November 29, 2023. Title: COMPOSITIONS AND METHODS FOR DETECTION OF ZIKA VIRUS. Applicant: Roche Diagnostics GmbH F. Hoffmann-La Roche AG Roche Molecular Systems, Inc. Application 62/306,803. The sequence listing filed with the application follows.

SEQUENCE LISTING (12 sequences)

SEQ ID NO: 1 - DNA, 21 bp, Artificial Sequence
  Primer
  modified_base (21)..(21): t-butylbenzyl dC
aacatggcggaggtaagatcc

SEQ ID NO: 2 - DNA, 20 bp, Artificial Sequence
  Primer
  modified_base (20)..(20): t-butylbenzyl dC
ctcccaccacttcaacaagc

SEQ ID NO: 3 - DNA, 21 bp, Artificial Sequence
  Primer
  modified_base (21)..(21): t-butylbenzyl dA
gaaccccaacaaacctggaga

SEQ ID NO: 4 - DNA, 26 bp, Artificial Sequence
  Primer
  modified_base (26)..(26): t-butylbenzyl dC
ttgtggatggaatagtggtaactgac

SEQ ID NO: 5 - DNA, 30 bp, Artificial Sequence
  Primer
  modified_base (30)..(30): t-butylbenzyl dC
taatgttcttttgcagacatattgagtgtc

SEQ ID NO: 6 - DNA, 19 bp, Artificial Sequence
  Primer
  modified_base (19)..(19): t-butylbenzyl dA
cagtctcccggatgctcca

SEQ ID NO: 7 - DNA, 26 bp, Artificial Sequence
  Primer
  modified_base (26)..(26): t-butylbenzyl dA
ctggaggtaaatgttgtcaagaagca

SEQ ID NO: 8 - DNA, 17 bp, Artificial Sequence
  Primer
  modified_base (17)..(17): t-butylbenzyl dC
agcctccccccatcccc

SEQ ID NO: 9 - DNA, 35 bp, Artificial Sequence
  Probe
tgcccaacacaaggtgaagcctaccttgacaagca

SEQ ID NO: 10 - DNA, 27 bp, Artificial Sequence
  Probe
ccgccaccaagatgaactgattggccg

SEQ ID NO: 11 - DNA, 33 bp, Artificial Sequence
  Probe
tggaggtgggtgtgcagagactgatgaagacca

SEQ ID NO: 12 - DNA, 42 bp, Artificial Sequence
  Probe
tgacacaatgacaattgacccccaagtggagaagaagatggg